European Patent Application EP 4 488 367 A1, published January 8, 2025. Title: 弹状病毒阴性草地贪夜蛾昆虫细胞株及其筛选、鉴定和应用. Applicant: 成都威斯克生物医药有限公司. Application CN. The sequence listing filed with the application follows.

SEQUENCE LISTING (11 sequences)

SEQ ID NO: 1 - DNA, 22 bp, synthetic construct
  source 1..22: mol_type = other DNA
aggagaactccaaagactcagc

SEQ ID NO: 2 - DNA, 20 bp, synthetic construct
  source 1..20: mol_type = other DNA
aaaaggagtccccactcagc

SEQ ID NO: 3 - DNA, 20 bp, synthetic construct
  source 1..20: mol_type = other DNA
ccacatctccgctatcacca

SEQ ID NO: 4 - DNA, 19 bp, synthetic construct
  source 1..19: mol_type = other DNA
aggagaaggagcggttgga

SEQ ID NO: 5 - DNA, 20 bp, synthetic construct
  source 1..20: mol_type = other DNA
tgaaaaccttcgcacagcac

SEQ ID NO: 6 - DNA, 20 bp, synthetic construct
  source 1..20: mol_type = other DNA
cgagacccctttggaccttt

SEQ ID NO: 7 - DNA, 20 bp, synthetic construct
  source 1..20: mol_type = other DNA
ggattgcacggagcctatca

SEQ ID NO: 8 - DNA, 20 bp, synthetic construct
  source 1..20: mol_type = other DNA
tgcccaagctaaggaaaggg

SEQ ID NO: 9 - DNA, 20 bp, synthetic construct
  source 1..20: mol_type = other DNA
tgacatgtggtctccaaccg

SEQ ID NO: 10 - DNA, 20 bp, synthetic construct
  source 1..20: mol_type = other DNA
gtatgcaggtggttgaggct

SEQ ID NO: 11 - DNA, 21 bp, synthetic construct
  source 1..21: mol_type = other DNA
ctccttctcctccacccacat